European Patent Specification EP 3 591 036 B1, published March 22, 2023. Title: METHODS OF DIFFERENTIATING STEM CELLS BY MODULATING MIR-124. Applicant: Accelerated BioSciences Corp. The sequence listing filed with the application follows.

SEQUENCE LISTING (158 sequences)

SEQ ID NO: 1 - RNA, 22 nt, Homo sapiens
cguguucacagcggaccuugau

SEQ ID NO: 2 - RNA, 20 nt, Homo sapiens
uaaggcacgcggugaaugcc

SEQ ID NO: 3 - RNA, 85 nt, Homo sapiens
aggccucucucuccguguucacagcggaccuugauuuaaauguccauacaauuaaggcacgcggugaaugccaagaauggggcug

SEQ ID NO: 4 - RNA, 19 nt, Aedes aegypti
uaaggcacgcggugaaugc

SEQ ID NO: 5 - RNA, 21 nt, Anolis carolinensis
uaaggcacgcggugaaugcca

SEQ ID NO: 6 - RNA, 21 nt, Anolis carolinensis
uaaggcacgcggugaaugcua

SEQ ID NO: 7 - RNA, 23 nt, Anopheles gambiae
uaaggcacgcggugaaugccaag

SEQ ID NO: 8 - RNA, 22 nt, Ateles geoffroyi
uuaaggcacgcggugaaugcca

SEQ ID NO: 9 - RNA, 23 nt, Apis mellifera
uaaggcacgcggugaaugccaag

SEQ ID NO: 10 - RNA, 21 nt, Acyrthosiphon pisum
uaaggcacgcggugaaugcca

SEQ ID NO: 11 - RNA, 22 nt, Ascaris suum
cgccuucaccggugacuuuggu

SEQ ID NO: 12 - RNA, 21 nt, Ascaris suum
uaaggcacgcggugaaugcca

SEQ ID NO: 13 - RNA, 22 nt, Branchiostoma floridae
aguguucacggcgguccuuaau

SEQ ID NO: 14 - RNA, 22 nt, Branchiostoma floridae
uaaggcacgcggugaaugccaa

SEQ ID NO: 15 - RNA, 22 nt, Brugia malayi
uaaggcacgcggugaaugccaa

SEQ ID NO: 16 - RNA, 23 nt, Bombyx mori
uaaggcacgcggugaaugccaag

SEQ ID NO: 17 - RNA, 23 nt, Bos taurus
uaaggcacgcggugaaugccaag

SEQ ID NO: 18 - RNA, 23 nt, Bos taurus
uaaggcacgcggugaaugccaag

SEQ ID NO: 19 - RNA, 21 nt, Caenorhabditis briggsae
uaaggcacgcggugaaugcca

SEQ ID NO: 20 - RNA, 20 nt, Cyprinus carpio
ucaagguccgcugugaacac

SEQ ID NO: 21 - RNA, 22 nt, Cyprinus carpio
ucaagguccgccgugaacacgc

SEQ ID NO: 22 - RNA, 23 nt, Caenorhabditis elegans
gcaugcacccuagugacuuuagu

SEQ ID NO: 23 - RNA, 21 nt, Caenorhabditis elegans
uaaggcacgcggugaaugcca

SEQ ID NO: 24 - RNA, 21 nt, Canis familiaris
uaaggcacgcggugaaugcca

SEQ ID NO: 25 - RNA, 21 nt, Canis familiaris
uaaggcacgcggugaaugcca

SEQ ID NO: 26 - RNA, 22 nt, Cricetulus griseus
uaaggcacgcggugaaugccaa

SEQ ID NO: 27 - RNA, 20 nt, Ciona intestinalis
aguauuuauuguggaccuug

SEQ ID NO: 28 - RNA, 22 nt, Ciona intestinalis
uaaggcacgcggugaaugccaa

SEQ ID NO: 29 - RNA, 20 nt, Ciona intestinalis
cguguuuacuguggaccuug

SEQ ID NO: 30 - RNA, 19 nt, Culex quinquefasciatus
uaaggcacgcggugaaugc

SEQ ID NO: 31 - RNA, 20 nt, Caenorhabditis remanei
uaaggcacgcggugaaugcc

SEQ ID NO: 32 - RNA, 22 nt, Ciona savignyi
uaaggcacgcggugaaugccaa

SEQ ID NO: 33 - RNA, 21 nt, Capitella teleta
uaaggcacgcggugaaugcca

SEQ ID NO: 34 - RNA, 23 nt, Drosophila ananassae
uaaggcacgcggugaaugccaag

SEQ ID NO: 35 - RNA, 23 nt, Drosophila erecta
uaaggcacgcggugaaugccaag

SEQ ID NO: 36 - RNA, 23 nt, Drosophila grimshawi
uaaggcacgcggugaaugccaag

SEQ ID NO: 37 - RNA, 23 nt, Drosophila melanogaster
gguauccacuguaggccuauaug

SEQ ID NO: 38 - RNA, 23 nt, Drosophila melanogaster
uaaggcacgcggugaaugccaag

SEQ ID NO: 39 - RNA, 23 nt, Drosophila mojavensis
uaaggcacgcggugaaugccaag

SEQ ID NO: 40 - RNA, 23 nt, Drosophila persimilis
uaaggcacgcggugaaugccaag

SEQ ID NO: 41 - RNA, 23 nt, Drosophila pseudoobscura
uaaggcacgcggugaaugccaag

SEQ ID NO: 42 - RNA, 23 nt, Daphnia pulex
uaaggcacgcggugaaugccaag

SEQ ID NO: 43 - RNA, 22 nt, Danio rerio
uaaggcacgcggugaaugccaa

SEQ ID NO: 44 - RNA, 23 nt, Drosophila sechellia
uaaggcacgcggugaaugccaag

SEQ ID NO: 45 - RNA, 23 nt, Drosophila simulans
uaaggcacgcggugaaugccaag

SEQ ID NO: 46 - RNA, 23 nt, Drosophila virilis
uaaggcacgcggugaaugccaag

SEQ ID NO: 47 - RNA, 23 nt, Drosophila willistoni
uaaggcacgcggugaaugccaag

SEQ ID NO: 48 - RNA, 23 nt, Drosophila yakuba
uaaggcacgcggugaaugccaag

SEQ ID NO: 49 - RNA, 20 nt, Equus caballus
uaaggcacgcggugaaugcc

SEQ ID NO: 50 - RNA, 21 nt, Echinococcus granulosus
uaaggcacgcggugaaugcca

SEQ ID NO: 51 - RNA, 23 nt, Echinococcus granulosus
guauucuacgcgaugucuuggua

SEQ ID NO: 52 - RNA, 20 nt, Echinococcus granulosus
uaaggcacgcggugaauacc

SEQ ID NO: 53 - RNA, 21 nt, Echinococcus multilocularis
uaaggcacgcggugaaugcca

SEQ ID NO: 54 - RNA, 20 nt, Echinococcus multilocularis
uaaggcacgcggugaauacc

SEQ ID NO: 55 - RNA, 22 nt, Fugu rubripes
uaaggcacgcggugaaugccaa

SEQ ID NO: 56 - RNA, 22 nt, Gallus gallus
uuaaggcacgcggugaaugcca

SEQ ID NO: 57 - RNA, 22 nt, Gallus gallus
uuaaggcacgcagugaaugcca

SEQ ID NO: 58 - RNA, 21 nt, Gallus gallus
cauucaccgcgugccuuaauu

SEQ ID NO: 59 - RNA, 22 nt, Gorilla gorilla
uuaaggcacgcggugaaugcca

SEQ ID NO: 60 - RNA, 22 nt, Haemonchus contortus
uaaggcacgcggugaaugccaa

SEQ ID NO: 61 - RNA, 22 nt, Heliconius melpomene
uaaggcacgcggugaaugccaa

SEQ ID NO: 62 - RNA, 23 nt, Ixodes scapularis
uaaggcacgcggugaaugccaag

SEQ ID NO: 63 - RNA, 21 nt, Lottia gigantean
uaaggcacgcggugaaugcca

SEQ ID NO: 64 - RNA, 22 nt, Lagothrix lagotricha
uuaaggcacgcggugaaugcca

SEQ ID NO: 65 - RNA, 22 nt, Monodelphis domestica
uuaaggcacgcggugaaugcca

SEQ ID NO: 66 - RNA, 22 nt, Macaca mulatta
uuaaggcacgcggugaaugcca

SEQ ID NO: 67 - RNA, 22 nt, Mus musculus
cguguucacagcggaccuugau

SEQ ID NO: 68 - RNA, 20 nt, Mus musculus
uaaggcacgcggugaaugcc

SEQ ID NO: 69 - RNA, 21 nt, Manduca sexta
uaaggcacgcggugaaugcca

SEQ ID NO: 70 - RNA, 23 nt, Nasonia vitripennis
uaaggcacgcggugaaugccaag

SEQ ID NO: 71 - RNA, 22 nt, Ornithorhynchus anatinus
cguguucacagcggaccuugau

SEQ ID NO: 72 - RNA, 21 nt, Ornithorhynchus anatinus
uaaggcacgcggugaaugcca

SEQ ID NO: 73 - RNA, 22 nt, Oikopleura dioica
uaaggcacgcggugaaugcuaa

SEQ ID NO: 74 - RNA, 22 nt, Oikopleura dioica
uaaggcacucggugaaugcuaa

SEQ ID NO: 75 - RNA, 19 nt, Oryzias latipes
cguguucacagcggaccuu

SEQ ID NO: 76 - RNA, 21 nt, Oryzias latipes
uaaggcacgcggugaaugcca

SEQ ID NO: 77 - RNA, 22 nt, Petromyzon marinus
cguguucacagcggaccuugau

SEQ ID NO: 78 - RNA, 21 nt, Petromyzon marinus
uaaggcacgcggugaaugcca

SEQ ID NO: 79 - RNA, 22 nt, Paralichthys olivaceus
cguguucacagcggaccuugau

SEQ ID NO: 80 - RNA, 22 nt, Paralichthys olivaceus
uaaggcacgcggugaaugccaa

SEQ ID NO: 81 - RNA, 22 nt, Pan paniscus
uuaaggcacgcggugaaugcca

SEQ ID NO: 82 - RNA, 20 nt, Pristionchus pacificus
uaaggcacgcggugaaugcc

SEQ ID NO: 83 - RNA, 20 nt, Pongo pygmaeus
uaaggcacgcggugaaugcc

SEQ ID NO: 84 - RNA, 22 nt, Pongo pygmaeus
uuaaggcacgcggugaaugcca

SEQ ID NO: 85 - RNA, 22 nt, Pan troglodytes
uuaaggcacgcggugaaugcca

SEQ ID NO: 86 - RNA, 22 nt, Rattus norvegicus
cguguucacagcggaccuugau

SEQ ID NO: 87 - RNA, 20 nt, Rattus norvegicus
uaaggcacgcggugaaugcc

SEQ ID NO: 88 - RNA, 25 nt, Schistosoma japonicum
ccauuuuccgcgauugccuugauuu

SEQ ID NO: 89 - RNA, 21 nt, Schistosoma japonicum
uaaggcacgcggugaauguca

SEQ ID NO: 90 - RNA, 22 nt, Saccoglossus kowalevskii
aguguucacagcgguccuugau

SEQ ID NO: 91 - RNA, 22 nt, Saccoglossus kowalevskii
uaaggcacgcggugaaugccaa

SEQ ID NO: 92 - RNA, 23 nt, Schmidtea mediterranea
ugcuuuuaacgcggagcuuuagu

SEQ ID NO: 93 - RNA, 21 nt, Schmidtea mediterranea
uaaggcacgcggugaaugcuu

SEQ ID NO: 94 - RNA, 23 nt, Schmidtea mediterranea
ugcauuuacaacgugucuuuagu

SEQ ID NO: 95 - RNA, 22 nt, Schmidtea mediterranea
uaaggcacgcggugaaugcuga

SEQ ID NO: 96 - RNA, 22 nt, Schmidtea mediterranea
gcgcucaccucgugaccuuugu

SEQ ID NO: 97 - RNA, 21 nt, Schmidtea mediterranea
uaaggcacgcggugaaugcca

SEQ ID NO: 98 - RNA, 23 nt, Schmidtea mediterranea
gcauuaacccuguugucuuagau

SEQ ID NO: 99 - RNA, 21 nt, Schmidtea mediterranea
gccauucucaguuggagucuu

SEQ ID NO: 100 - RNA, 21 nt, Schmidtea mediterranea
uaaggcacgcugugaaugcca

SEQ ID NO: 101 - RNA, 21 nt, Strongylocentrotus purpuratus
uaaggcacgcggugaaugcca

SEQ ID NO: 102 - RNA, 21 nt, Sus scrofa
uaaggcacgcggugaaugcca

SEQ ID NO: 103 - RNA, 21 nt, Sus scrofa
uaaggcacgcggugaaugcca

SEQ ID NO: 104 - RNA, 22 nt, Tribolium castaneu
aguguucacuguuggccuguau

SEQ ID NO: 105 - RNA, 23 nt, Tribolium castaneu
uaaggcacgcggugaaugccaag

SEQ ID NO: 106 - RNA, 21 nt, Taeniopygia guttata
cguguucacagcggaccuuga

SEQ ID NO: 107 - RNA, 21 nt, Taeniopygia guttata
uaaggcacgcggugaaugcca

SEQ ID NO: 108 - RNA, 22 nt, Tetraodon nigroviridis
uaaggcacgcggugaaugccaa

SEQ ID NO: 109 - RNA, 22 nt, Tetranychus urticae
cguguucacuguguaugucuug

SEQ ID NO: 110 - RNA, 21 nt, Tetranychus urticae
uaaggcacgcggugaaugcca

SEQ ID NO: 111 - RNA, 22 nt, Tetranychus urticae
guguucacuguuugccuucaug

SEQ ID NO: 112 - RNA, 22 nt, Xenoturbella bocki
uaaggcacgcggugaaugccaa

SEQ ID NO: 113 - RNA, 22 nt, Xenopus tropicalis
uuaaggcacgcggugaaugcca

SEQ ID NO: 114 - RNA, 21 nt, Schmidtea mediterranea
uaaggcacgcgguaagugggu

SEQ ID NO: 115 - RNA, 23 nt, Schmidtea mediterranea
aacauuuacaagcgagccuuaau

SEQ ID NO: 116 - DNA, 21 bp, Artificial Sequence
  Description of Artificial Sequence: Synthetic oligonucleotide
gtacttcataccatgccgatt

SEQ ID NO: 117 - DNA, 58 bp, Artificial Sequence
  Description of Artificial Sequence: Synthetic oligonucleotide
ccgggtacttcataccatgccgattctcgagaatcggcatggtatgaagtactttttg

SEQ ID NO: 118 - DNA, 21 bp, Artificial Sequence
  Description of Artificial Sequence: Synthetic oligonucleotide
cagattgtcttgcaacttcag

SEQ ID NO: 119 - DNA, 58 bp, Artificial Sequence
  Description of Artificial Sequence: Synthetic oligonucleotide
ccggcagattgtcttgcaacttcagctcgagctgaagttgcaagacaatctgtttttg

SEQ ID NO: 120 - DNA, 21 bp, Artificial Sequence
  Description of Artificial Sequence: Synthetic oligonucleotide
taccatacagagaacattgga

SEQ ID NO: 121 - DNA, 58 bp, Artificial Sequence
  Description of Artificial Sequence: Synthetic oligonucleotide
ccggtaccatacagagaacattggactcgagtccaatgttctctgtatggtatttttg

SEQ ID NO: 122 - DNA, 20 bp, Artificial Sequence
  Description of Artificial Sequence: Synthetic primer
acatctccctccccagactc

SEQ ID NO: 123 - DNA, 20 bp, Artificial Sequence
  Description of Artificial Sequence: Synthetic primer
tgctctgtgctcagaagtgg

SEQ ID NO: 124 - DNA, 21 bp, Artificial Sequence
  Description of Artificial Sequence: Synthetic primer
ctgtcggctgagggtttccat

SEQ ID NO: 125 - DNA, 20 bp, Artificial Sequence
  Description of Artificial Sequence: Synthetic primer
gagtctggggagggagatgt

SEQ ID NO: 126 - DNA, 20 bp, Artificial Sequence
  Description of Artificial Sequence: Synthetic primer
tctgcggctctttggtttca

SEQ ID NO: 127 - DNA, 20 bp, Artificial Sequence
  Description of Artificial Sequence: Synthetic primer
tctgccttcagcacaagagg

SEQ ID NO: 128 - DNA, 20 bp, Artificial Sequence
  Description of Artificial Sequence: Synthetic primer
gcggctctttggtttcaagg

SEQ ID NO: 129 - DNA, 20 bp, Artificial Sequence
  Description of Artificial Sequence: Synthetic primer
ctgccttcagcacaagagga

SEQ ID NO: 130 - DNA, 20 bp, Artificial Sequence
  Description of Artificial Sequence: Synthetic primer
cccgcagttctcaaggacac

SEQ ID NO: 131 - DNA, 20 bp, Artificial Sequence
  Description of Artificial Sequence: Synthetic primer
agaagggagccaggcaagtc

SEQ ID NO: 132 - DNA, 23 bp, Artificial Sequence
  Description of Artificial Sequence: Synthetic primer
ttgtagattgctctctctcctcc

SEQ ID NO: 133 - DNA, 19 bp, Artificial Sequence
  Description of Artificial Sequence: Synthetic primer
gtgaagccttggctagggg

SEQ ID NO: 134 - DNA, 20 bp, Artificial Sequence
  Description of Artificial Sequence: Synthetic primer
cccatcattgattcctggat

SEQ ID NO: 135 - DNA, 20 bp, Artificial Sequence
  Description of Artificial Sequence: Synthetic primer
ttgggaggctgagatttgtc

SEQ ID NO: 136 - DNA, 20 bp, Artificial Sequence
  Description of Artificial Sequence: Synthetic primer
gtcagccctccctgactgat

SEQ ID NO: 137 - DNA, 20 bp, Artificial Sequence
  Description of Artificial Sequence: Synthetic primer
catgtggatttccagcctgc

SEQ ID NO: 138 - DNA, 29 bp, Artificial Sequence
  Description of Artificial Sequence: Synthetic primer
aaattataagctgtttgggttgttggtct

SEQ ID NO: 139 - DNA, 29 bp, Artificial Sequence
  Description of Artificial Sequence: Synthetic primer
aaacaattgcccccataatttctgactgc

SEQ ID NO: 140 - DNA, 29 bp, Artificial Sequence
  Description of Artificial Sequence: Synthetic primer
aaattataactcccaaagtgctgggatta

SEQ ID NO: 141 - DNA, 29 bp, Artificial Sequence
  Description of Artificial Sequence: Synthetic primer
aaacaattgctgcactgttcacaggagga

SEQ ID NO: 142 - DNA, 29 bp, Artificial Sequence
  Description of Artificial Sequence: Synthetic primer
aaattataacagttgtcccagtgctgcta

SEQ ID NO: 143 - DNA, 29 bp, Artificial Sequence
  Description of Artificial Sequence: Synthetic primer
aaacaattgatgacttgcccaaaggtcac

SEQ ID NO: 144 - DNA, 29 bp, Artificial Sequence
  Description of Artificial Sequence: Synthetic primer
aaattataacccacaactggggtaaaaga

SEQ ID NO: 145 - DNA, 29 bp, Artificial Sequence
  Description of Artificial Sequence: Synthetic primer
aaacaattgctgtggaaggggcaaagata

SEQ ID NO: 146 - RNA, 109 nt, Homo sapiens
aucaagauuagaggcucugcucuccguguucacagcggaccuugauuuaaugucauacaauuaaggcacgcggugaaugccaagagcggagccuacggcugcacuugaa

SEQ ID NO: 147 - RNA, 87 nt, Homo sapiens
ugagggccccucugcguguucacagcggaccuugauuuaaugucuauacaauuaaggcacgcggugaaugccaagagaggcgccucc

SEQ ID NO: 148 - DNA, 11 bp, Unknown
  Description of Unknown: CREB1-binding site 1 oligonucleotide
acgccgtcatt

SEQ ID NO: 149 - DNA, 12 bp, Unknown
  Description of Unknown: CREB1-binding site 2 oligonucleotide
ggtgacgtcagc

SEQ ID NO: 150 - DNA, 12 bp, Unknown
  Description of Unknown: CREB1-binding site oligonucleotide
ggtgacgtcacc

SEQ ID NO: 151 - RNA, 17 nt, Homo sapiens
guuuguccagugccuuu

SEQ ID NO: 152 - RNA, 16 nt, Homo sapiens
auccagaauugccuua

SEQ ID NO: 153 - RNA, 17 nt, Homo sapiens
gggaguauuugaacaca

SEQ ID NO: 154 - RNA, 17 nt, Homo sapiens
cguguucacagcggacc

SEQ ID NO: 155 - RNA, 15 nt, Homo sapiens
guuuggagugccuuc

SEQ ID NO: 156 - RNA, 15 nt, Homo sapiens
uaaggcacgcgguga

SEQ ID NO: 157 - DNA, 16 bp, Unknown
  Description of Unknown: Foxa2 oligonucleotide
cctgtttgttttagtt

SEQ ID NO: 158 - DNA, 8 bp, Unknown
  Description of Unknown: Cis-regulatory element (CRE) oligonucleotide
tgacgtca